European Patent Specification EP 3 817 773 B1, published July 24, 2024. Title: HUMANIZED ANTIBODIES AGAINST C-KIT. Applicant: FORTY SEVEN, INC. LIU, JIE SOMPALLI, KAVITHA. The sequence listing filed with the application follows.

SEQUENCE LISTING (54 sequences)

SEQ ID NO: 1 - protein, 117 aa, Artificial sequence
  Synthesized
QVQLQQPGAELVKPGASVKMSCKASGYTFTSYNMHWVKQTPGQGLEWIGVIYSGNGDTSYNQKFKGKATLTADKSSSTAYMQINSLTSEDSAVYYCARERDTRFGNWGQGTLVTVSA

SEQ ID NO: 2 - protein, 5 aa, Artificial sequence
  Synthesized
SYNMH

SEQ ID NO: 3 - protein, 17 aa, Artificial sequence
  Synthesized
VIYSGNGDTSYNQKFKG

SEQ ID NO: 4 - protein, 8 aa, Artificial sequence
  Synthesized
ERDTRFGN

SEQ ID NO: 5 - protein, 111 aa, Artificial sequence
  Synthesized
NIVLTQSPASLAVSLGLRATISCRASESVDIYGNSFMHWYQQKPGQPPKLLIYLASNLESGVPARFSGSGSRTDFTLTIDPVEADDAATYYCQQNNEDPYTFGGGTKLEIK

SEQ ID NO: 6 - protein, 15 aa, Artificial sequence
  Synthesized
RASESVDIYGNSFMH

SEQ ID NO: 7 - protein, 7 aa, Artificial sequence
  Synthesized
LASNLES

SEQ ID NO: 8 - protein, 9 aa, Artificial sequence
  Synthesized
QQNNEDPYT

SEQ ID NO: 9 - protein, 117 aa, Artificial sequence
  Synthesized
QVQLVQSGAEVKKPGASVKVSCKASGYTFTSYNMHWVRQAPGQGLEWMGVIYSGQGDTSYNQKFKGRVTITADKSTSTAYMELSSLRSEDTAVYYCARERDTRFGNWGQGTLVTVSS

SEQ ID NO: 10 - protein, 5 aa, Artificial sequence
  Synthesized
SYNMH

SEQ ID NO: 11 - protein, 17 aa, Artificial sequence
  Synthesized
VIYSGQGDTSYNQKFKG

SEQ ID NO: 12 - protein, 8 aa, Artificial sequence
  Synthesized
ERDTRFGN

SEQ ID NO: 13 - protein, 117 aa, Artificial sequence
  Synthesized
QVQLVQSGAEVKKPGASVKVSCKASGYTFTSYNMHWVRQAPGQGLEWMGVIYSGNGDTSYAQKFKGRVTITADKSTSTAYMELSSLRSEDTAVYYCARERDTRFGNWGQGTLVTVSS

SEQ ID NO: 14 - protein, 5 aa, Artificial sequence
  Synthesized
SYNMH

SEQ ID NO: 15 - protein, 17 aa, Artificial sequence
  Synthesized
VIYSGNGDTSYAQKFKG

SEQ ID NO: 16 - protein, 8 aa, Artificial sequence
  Synthesized
ERDTRFGN

SEQ ID NO: 17 - protein, 117 aa, Artificial sequence
  Synthesized
QVQLVQSGAEVKKPGASVKVSCKASGYTFTSYNMHWVRQAPGQGLEWMGVIYSGNGDTSYNQKFQGRVTITADKSTSTAYMELSSLRSEDTAVYYCARERDTRFGNWGQGTLVTVSS

SEQ ID NO: 18 - protein, 5 aa, Artificial sequence
  Synthesized
SYNMH

SEQ ID NO: 19 - protein, 17 aa, Artificial sequence
  Synthesized
VIYSGNGDTSYNQKFQG

SEQ ID NO: 20 - protein, 8 aa, Artificial sequence
  Synthesized
ERDTRFGN

SEQ ID NO: 21 - protein, 117 aa, Artificial sequence
  Synthesized
QVQLVQSGAEVKKPGASVKVSCKASGYTFTSYNMHWVRQAPGQGLEWMGVIYSGNGDTSYAQKFQGRVTITADKSTSTAYMELSSLRSEDTAVYYCARERDTRFGNWGQGTLVTVSS

SEQ ID NO: 22 - protein, 5 aa, Artificial sequence
  Synthesized
SYNMH

SEQ ID NO: 23 - protein, 17 aa, Artificial sequence
  Synthesized
VIYSGNGDTSYAQKFQG

SEQ ID NO: 24 - protein, 8 aa, Artificial sequence
  Synthesized
ERDTRFGN

SEQ ID NO: 25 - protein, 117 aa, Artificial sequence
  Synthesized
QVQLVQSGAEVKKPGASVKVSCKASGYTFTSYNMHWVRQAPGQGLEWMGVIYSGNGDTSYNQKFKGRVTITADKSTSTAYMELSSLRSEDTAVYYCARDRDTRFGNWGQGTLVTVSS

SEQ ID NO: 26 - protein, 5 aa, Artificial sequence
  Synthesized
SYNMH

SEQ ID NO: 27 - protein, 17 aa, Artificial sequence
  Synthesized
VIYSGNGDTSYNQKFKG

SEQ ID NO: 28 - protein, 8 aa, Artificial sequence
  Synthesized
DRDTRFGN

SEQ ID NO: 29 - protein, 117 aa, Artificial sequence
  Synthesized
QVQLVQSGAEVKKPGASVKVSCKASGYTFTSYNMHWVRQAPGQGLEWMGVIYSGNGDTSYNQKFKGRVTITADKSTSTAYMELSSLRSEDTAVYYCARERDTRFGNWGQGTLVTVSS

SEQ ID NO: 30 - protein, 98 aa, Homo sapiens
QVQLVQSGAEVKKPGASVKVSCKASGYTFTSYYMHWVRQAPGQGLEWMGIINPSGGSTSYAQKFQGRVTMTRDTSTSTVYMELSSLRSEDTAVYYCAR

SEQ ID NO: 31 - protein, 111 aa, Artificial sequence
  Synthesized
DIVMTQSPDSLAVSLGERATINCRASDSVDIYGNSFMHWYQQKPGQPPKLLIYLASNLESGVPDRFSGSGSGTDFTLTISSLQAEDVAVYYCQQNNEDPYTFGGGTKVEIK

SEQ ID NO: 32 - protein, 15 aa, Artificial sequence
  Synthesized
RASDSVDIYGNSFMH

SEQ ID NO: 33 - protein, 7 aa, Artificial sequence
  Synthesized
LASNLES

SEQ ID NO: 34 - protein, 9 aa, Artificial sequence
  Synthesized
QQNNEDPYT

SEQ ID NO: 35 - protein, 111 aa, Artificial sequence
  Synthesized
DIVMTQSPDSLAVSLGERATINCRASESVDIYGQSFMHWYQQKPGQPPKLLIYLASNLESGVPDRFSGSGSGTDFTLTISSLQAEDVAVYYCQQNNEDPYTFGGGTKVEIK

SEQ ID NO: 36 - protein, 15 aa, Artificial sequence
  Synthesized
RASESVDIYGQSFMH

SEQ ID NO: 37 - protein, 7 aa, Artificial sequence
  Synthesized
LASNLES

SEQ ID NO: 38 - protein, 9 aa, Artificial sequence
  Synthesized
QQNNEDPYT

SEQ ID NO: 39 - protein, 111 aa, Artificial sequence
  Synthesized
DIVMTQSPDSLAVSLGERATINCRASESVDIYGNSFMHWYQQKPGQPPKLLIYLASNLESGVPDRFSGSGSGTDFTLTISSLQAEDVAVYYCQQNNEDPYTFGGGTKVEIK

SEQ ID NO: 40 - protein, 101 aa, Homo sapiens
DIVMTQSPDSLAVSLGERATINCKSSQSVLYSSNNKNYLAWYQQKPGQPPKLLIYWASTRESGVPDRFSGSGSGTDFTLTISSLQAEDVAVYYCQQYYSTP

SEQ ID NO: 41 - protein, 17 aa, Homo sapiens
KSSQSVLYSSNNKNYLA

SEQ ID NO: 42 - protein, 7 aa, Homo sapiens
WASTRES

SEQ ID NO: 43 - protein, 7 aa, Homo sapiens
QQYYSTP

SEQ ID NO: 44 - protein, 117 aa, Artificial sequence
  Synthesized
EVQLLESGGGLVQPGGSLRLSCAASGFTFTSYNMHWVRQAPGKGLEWVGVIYSGNGDTSYNQKFKGRFTISADKSKNTAYLQMNSLRAEDTAVYYCARERDTRFGNWGQGTLVTVSS

SEQ ID NO: 45 - protein, 117 aa, Artificial sequence
  Synthesized
EVQLLESGGGLVQPGGSLRLSCAASGFTFTSYNMHWVRQAPGKGLEWVGVIYSGQGDTSYNQKFKGRFTISADKSKNTAYLQMNSLRAEDTAVYYCARERDTRFGNWGQGTLVTVSS

SEQ ID NO: 46 - protein, 117 aa, Artificial sequence
  Synthesized
EVQLLESGGGLVQPGGSLRLSCAASGFTFTSYNMHWVRQAPGKGLEWVGVIYSGNGDTSYAQKFKGRFTISADKSKNTAYLQMNSLRAEDTAVYYCARERDTRFGNWGQGTLVTVSS

SEQ ID NO: 47 - protein, 117 aa, Artificial sequence
  Synthesized
EVQLLESGGGLVQPGGSLRLSCAASGFTFTSYNMHWVRQAPGKGLEWVGVIYSGNGDTSYNQKFQGRFTISADKSKNTAYLQMNSLRAEDTAVYYCARERDTRFGNWGQGTLVTVSS

SEQ ID NO: 48 - protein, 117 aa, Artificial sequence
  Synthesized
EVQLLESGGGLVQPGGSLRLSCAASGFTFTSYNMHWVRQAPGKGLEWVGVIYSGNGDTSYAQKFQGRFTISADKSKNTAYLQMNSLRAEDTAVYYCARERDTRFGNWGQGTLVTVSS

SEQ ID NO: 49 - protein, 117 aa, Artificial sequence
  Synthesized
EVQLLESGGGLVQPGGSLRLSCAASGFTFTSYNMHWVRQAPGKGLEWVGVIYSGNGDTSYNQKFKGRFTISADKSKNTAYLQMNSLRAEDTAVYYCARDRDTRFGNWGQGTLVTVSS

SEQ ID NO: 50 - protein, 98 aa, Homo sapiens
EVQLLESGGGLVQPGGSLRLSCAASGFTFSSYAMSWVRQAPGKGLEWVSAISGSGGSTYYADSVKGRFTISRDNSKNTLYLQMNSLRAEDTAVYYCAK

SEQ ID NO: 51 - protein, 111 aa, Artificial sequence
  Synthesized
DIVMTQSPLSLPVTPGEPASISCRASESVDIYGNSFMHWYLQKPGQSPQLLIYLASNLESGVPDRFSGSGSGTDFTLKISRVEAEDVGVYYCQQNNEDPYTFGGGTKVEIK

SEQ ID NO: 52 - protein, 111 aa, Artificial sequence
  Synthesized
DIVMTQSPLSLPVTPGEPASISCRASDSVDIYGNSFMHWYLQKPGQSPQLLIYLASNLESGVPDRFSGSGSGTDFTLKISRVEAEDVGVYYCQQNNEDPYTFGGGTKVEIK

SEQ ID NO: 53 - protein, 111 aa, Artificial sequence
  Synthesized
DIVMTQSPLSLPVTPGEPASISCRASESVDIYGQSFMHWYLQKPGQSPQLLIYLASNLESGVPDRFSGSGSGTDFTLKISRVEAEDVGVYYCQQNNEDPYTFGGGTKVEIK

SEQ ID NO: 54 - protein, 100 aa, Homo sapiens
DIVMTQSPLSLPVTPGEPASISCRSSQSLLHSNGYNYLDWYLQKPGQSPQLLIYLGSNRASGVPDRFSGSGSGTDFTLKISRVEAEDVGVYYCMQALQTP